European Patent Specification EP 3 849 614 B1, published December 20, 2023. Title: Interleukin-2 Polypeptide Conjugates and Their Uses. Applicant: Ambrx, Inc. The sequence listing filed with the application follows.

SEQUENCE LISTING (23 sequences)

SEQ ID NO: 1 - protein, 153 aa, Human
MYRMQLLSCIALSLALVTNSAPTSSSTKKTQLQLEHLLLDLQMILNGINNYKNPKLTRMLTFKFYMPKKATELKHLQCLEEELKPLEEVLNLAQSKNFHLRPRDLISNINVIVLELKGSETTFMCEYADETATIVEFLNRWITFCQSIISTLT

SEQ ID NO: 2 - protein, 133 aa, Human [sequence omitted]

SEQ ID NO: 3 - protein, 133 aa, E. Coli [sequence omitted]

SEQ ID NO: 4 - DNA, 399 bp, E. Coli
atgccgaccagcagtagcaccaagaaaactcagctgcagctggagcatctgctgctggatttacagatgattctgaatggcattaataattacaaaaatccgaaactgacccgcatgctgaccttcaagttctacatgccgaagaaggccaccgaactgaagcatctgcagtgtttagaagaggaactgaagccgctggaagaggtgctgaatttagcccagagcaaaaacttccatctgcgcccgcgcgatttaattagcaatattaacgtgattgtgctggaactgaaaggcagcgagaccacctttatgtgcgagtacgcagatgagaccgccaccatcgtggaatttttaaaccgctggatcaccttcagccagagtatcattagcactttaacc

SEQ ID NO: 5 - protein, 134 aa, E. Coli
MAPTSSSTKKTQLQLEHLLLDLQMILNGINNYKNPKLTRMLTFKFYMPKKATELKHLQCLEEELKPLEEVLNLAQSKNFHLRPRDLISNINVIVLELKGSETTFMCEYADETATIVEFLNRWITFSQSIISTLT

SEQ ID NO: 6 - DNA, 402 bp, Human
atggcaccgaccagcagtagcaccaagaaaactcagctgcagctggagcatctgctgctggatttacagatgattctgaatggcattaataattacaaaaatccgaaactgacccgcatgctgaccttcaagttctacatgccgaagaaggccaccgaactgaagcatctgcagtgtttagaagaggaactgaagccgctggaagaggtgctgaatttagcccagagcaaaaacttccatctgcgcccgcgcgatttaattagcaatattaacgtgattgtgctggaactgaaaggcagcgagaccacctttatgtgcgagtacgcagatgagaccgccaccatcgtggaatttttaaaccgctggatcaccttcagccagagtatcattagcactttaacc

SEQ ID NO: 7 - protein, 132 aa, Human
MTSSSTKKTQLQLEHLLLDLQMILNGINNYKNPKLTRMLTFKFYMPKKATELKHLQCLEEELKPLEEVLNLAQSKNFHLRPRDLISNINVIVLELKGSETTFMCEYADETATIVEFLNRWITFSQSIISTLT

SEQ ID NO: 8 - DNA, 396 bp, Human
atgaccagcagtagcaccaagaaaactcagctgcagctggagcatctgctgctggatttacagatgattctgaatggcattaataattacaaaaatccgaaactgacccgcatgctgaccttcaagttctacatgccgaagaaggccaccgaactgaagcatctgcagtgtttagaagaggaactgaagccgctggaagaggtgctgaatttagcccagagcaaaaacttccatctgcgcccgcgcgatttaattagcaatattaacgtgattgtgctggaactgaaaggcagcgagaccacctttatgtgcgagtacgcagatgagaccgccaccatcgtggaatttttaaaccgctggatcaccttcagccagagtatcattagcactttaacc

SEQ ID NO: 9 - protein, 133 aa, Human
  misc_feature (42)..(42): Xaa = *U = Unnatural Amino Acid
APTSSSTKKTQLQLEHLLLDLQMILNGINNYKNPKLTRMLTXKFYMPKKATELKHLQCLEEELKPLEEVLNLAQSKNFHLRPRDLISNINVIVLELKGSETTFMCEYADETATIVEFLNRWITFCQSIISTLT

SEQ ID NO: 10 - protein, 133 aa, Human
  misc_feature (44)..(44): Xaa = *U = Unnatural Amino Acid
APTSSSTKKTQLQLEHLLLDLQMILNGINNYKNPKLTRMLTFKXYMPKKATELKHLQCLEEELKPLEEVLNLAQSKNFHLRPRDLISNINVIVLELKGSETTFMCEYADETATIVEFLNRWITFCQSIISTLT

SEQ ID NO: 11 - protein, 133 aa, Human
  misc_feature (45)..(45): Xaa = *U = Unnatural Amino Acid
APTSSSTKKTQLQLEHLLLDLQMILNGINNYKNPKLTRMLTFKFXMPKKATELKHLQCLEEELKPLEEVLNLAQSKNFHLRPRDLISNINVIVLELKGSETTFMCEYADETATIVEFLNRWITFCQSIISTLT

SEQ ID NO: 12 - protein, 133 aa, Human
  misc_feature (65)..(65): Xaa = *U = Unnatural Amino Acid
APTSSSTKKTQLQLEHLLLDLQMILNGINNYKNPKLTRMLTFKFYMPKKATELKHLQCLEEELKXLEEVLNLAQSKNFHLRPRDLISNINVIVLELKGSETTFMCEYADETATIVEFLNRWITFCQSIISTLT

SEQ ID NO: 13 - protein, 133 aa, Human
  misc_feature (72)..(72): Xaa = *U = Unnatural Amino Acid
APTSSSTKKTQLQLEHLLLDLQMILNGINNYKNPKLTRMLTFKFYMPKKATELKHLQCLEEELKPLEEVLNXAQSKNFHLRPRDLISNINVIVLELKGSETTFMCEYADETATIVEFLNRWITFCQSIISTLT

SEQ ID NO: 14 - protein, 133 aa, Human
  misc_feature (61)..(61): Xaa = *U = Unnatural Amino Acid
APTSSSTKKTQLQLEHLLLDLQMILNGINNYKNPKLTRMLTFKFYMPKKATELKHLQCLEXELKPLEEVLNLAQSKNFHLRPRDLISNINVIVLELKGSETTFMCEYADETATIVEFLNRWITFCQSIISTLT

SEQ ID NO: 15 - protein, 133 aa, Human
  misc_feature (62)..(62): Xaa = *U = Unnatural Amino Acid
  misc_feature (68)..(68): Xaa = U = Unnatural Amino Acid
APTSSSTKKTQLQLEHLLLDLQMILNGINNYKNPKLTRMLTFKFYMPKKATELKHLQCLEEXLKPLEXVLNLAQSKNFHLRPRDLISNINVIVLELKGSETTFMCEYADETATIVEFLNRWITFCQSIISTLT

SEQ ID NO: 16 - protein, 133 aa, Human
  misc_feature (35)..(35): Xaa = *U = Unnatural Amino Acid
APTSSSTKKTQLQLEHLLLDLQMILNGINNYKNPXLTRMLTFKFYMPKKATELKHLQCLEEELKPLEEVLNLAQSKNFHLRPRDLISNINVIVLELKGSETTFMCEYADETATIVEFLNRWITFCQSIISTLT

SEQ ID NO: 17 - protein, 133 aa, Human
  misc_feature (38)..(38): Xaa = *U = Unnatural Amino Acid
APTSSSTKKTQLQLEHLLLDLQMILNGINNYKNPKLTXMLTFKFYMPKKATELKHLQCLEEELKPLEEVLNLAQSKNFHLRPRDLISNINVIVLELKGSETTFMCEYADETATIVEFLNRWITFCQSIISTLT

SEQ ID NO: 18 - protein, 133 aa, Human
  misc_feature (43)..(43): Xaa = *U = Unnatural Amino Acid
APTSSSTKKTQLQLEHLLLDLQMILNGINNYKNPKLTRMLTFXFYMPKKATELKHLQCLEEELKPLEEVLNLAQSKNFHLRPRDLISNINVIVLELKGSETTFMCEYADETATIVEFLNRWITFCQSIISTLT

SEQ ID NO: 19 - protein, 133 aa, Human
  misc_feature (37)..(37): Xaa = *U = Unnatural Amino Acid
APTSSSTKKTQLQLEHLLLDLQMILNGINNYKNPKLXRMLTFKFYMPKKATELKHLQCLEEELKPLEEVLNLAQSKNFHLRPRDLISNINVIVLELKGSETTFMCEYADETATIVEFLNRWITFCQSIISTLT

SEQ ID NO: 20 - protein, 133 aa, Human
  misc_feature (3)..(3): Xaa = *U = Unnatural Amino Acid
APXSSSTKKTQLQLEHLLLDLQMILNGINNYKNPKLTRMLTFKFYMPKKATELKHLQCLEEELKPLEEVLNLAQSKNFHLRPRDLISNINVIVLELKGSETTFMCEYADETATIVEFLNRWITFCQSIISTLT

SEQ ID NO: 21 - protein, 133 aa, Human
  misc_feature (64)..(64): Xaa = *U = Unnatural Amino Acid
APTSSSTKKTQLQLEHLLLDLQMILNGINNYKNPKLTRMLTFKFYMPKKATELKHLQCLEEELXPLEEVLNLAQSKNFHLRPRDLISNINVIVLELKGSETTFMCEYADETATIVEFLNRWITFCQSIISTLT

SEQ ID NO: 22 - protein, 133 aa, Human
  misc_feature (68)..(68): Xaa = *U = Unnatural Amino Acid
APTSSSTKKTQLQLEHLLLDLQMILNGINNYKNPKLTRMLTFKFYMPKKATELKHLQCLEEELKPLEXVLNLAQSKNFHLRPRDLISNINVIVLELKGSETTFMCEYADETATIVEFLNRWITFCQSIISTLT

SEQ ID NO: 23 - protein, 133 aa, Human
  misc_feature (107)..(107): Xaa = *U = Unnatural Amino Acid
APTSSSTKKTQLQLEHLLLDLQMILNGINNYKNPKLTRMLTFKFYMPKKATELKHLQCLEEELKPLEEVLNLAQSKNFHLRPRDLISNINVIVLELKGSETTFMCEXADETATIVEFLNRWITFCQSIISTLT